European Patent Specification EP 4 029 515 B1, published December 4, 2024. Title: ANTI-INFECTION EFFECTS OF HNRNPA2B1 AND USE THEREOF. Applicant: INSTITUTE OF BASIC MEDICAL SCIENCES, CHINESE ACADEMY OF MEDICAL SCIENCES. The sequence listing filed with the application follows.

SEQUENCE LISTING (10 sequences)

SEQ ID NO: 1 - DNA, 1026 bp, Homo sapiens
atggagagagaaaaggaacagttccgtaagctctttattggtggcttaagctttgaaaccacagaagaaagtttgaggaactactacgaacaatggggaaagcttacagactgtgtggtaatgagggatcctgcaagcaaaagatcaagaggatttggttttgtaactttttcatccatggctgaggttgatgctgccatggctgcaagacctcattcaattgatgggagagtagttgagccaaaacgtgctgtagcaagagaggaatctggaaaaccaggggctcatgtaactgtgaagaagctgtttgttggcggaattaaagaagatactgaggaacatcaccttagagattactttgaggaatatggaaaaattgataccattgagataattactgataggcagtctggaaagaaaagaggctttggctttgttacttttgatgaccatgatcctgtggataaaatcgtattgcagaaataccataccatcaatggtcataatgcagaagtaagaaaggctttgtctagacaagaaatgcaggaagttcagagttctaggagtggaagaggaggcaactttggctttggggattcacgtggtggcggtggaaatttcggaccaggaccaggaagtaactttagaggaggatctgatggatatggcagtggacgtggatttggggatggctataatgggtatggaggaggacctggaggtggcaattttggaggtagccccggttatggaggaggaagaggaggatatggtggtggaggacctggatatggcaaccagggtgggggctacggaggtggttatgacaactatggaggaggaaattatggaagtggaaattacaatgattttggaaattataaccagcaaccttctaactacggtccaatgaagagtggaaactttggtggtagcaggaacatggggggaccatatggtggaggaaactatggtccaggaggcagtggaggaagtgggggttatggtgggaggagccgatactga

SEQ ID NO: 2 - protein, 341 aa, Homo sapiens
MEREKEQFRKLFIGGLSFETTEESLRNYYEQWGKLTDCVVMRDPASKRSRGFGFVTFSSMAEVDAAMAARPHSIDGRVVEPKRAVAREESGKPGAHVTVKKLFVGGIKEDTEEHHLRDYFEEYGKIDTIEIITDRQSGKKRGFGFVTFDDHDPVDKIVLQKYHTINGHNAEVRKALSRQEMQEVQSSRSGRGGNFGFGDSRGGGGNFGPGPGSNFRGGSDGYGSGRGFGDGYNGYGGGPGGGNFGGSPGYGGGRGGYGGGGPGYGNQGGGYGGGYDNYGGGNYGSGNYNDFGNYNQQPSNYGPMKSGNFGGSRNMGGPYGGGNYGPGGSGGSGGYGGRSRY

SEQ ID NO: 3 - DNA, 906 bp, Mus musculus
atggagagagaaaaggaacagttccgaaagctctttattggtggcttaagctttgaaaccacagaagaaagtttgagaaactactatgagcaatggggaaagctcacagactgtgtggttatgcgggatcctgcaagcaaaagatcaagaggatttggctttgtaactttctcatccatggccgaggttgacgctgccatggctgcaaggccccattccattgatggcagggtagttgagccaaaacgtgctgtagcaagagaggagtctggaaaaccaggagcccatgtgactgtgaagaagctgtttgttggtggaattaaggaagatactgaggaacaccaccttagagattactttgaagagtatggaaaaattgatactattgaaataattaccgataggcagtctggaaagaaaagaggctttggctttgttacttttgatgaccatgatcctgtggataaaattgtcttgcaaaaatatcacaccataaatggtcacaatgcagaagttagaaaggcattgtctagacaagaaatgcaggaagtccaaagttctaggagtggaagaggaggaaactttggttttggggattctcgtggtggcggtggcaattttggaccaggaccaggaagcaactttagggggggatctgatggatacggaagtggacgtggatttggggatggctataatgggtatggaggaggacctggaggaaattatggaagtggaagttacaatgattttggaaattataaccagcagccttctaactatggtccaatgaagagtggaaactttgggggtagcaggaacatgggaggaccatatggtggagggaactatggtcctggaggaagtggaggaagtggtggctatggtggaaggagcagatattaa

SEQ ID NO: 4 - protein, 301 aa, Mus musculus
MEREKEQFRKLFIGGLSFETTEESLRNYYEQWGKLTDCVVMRDPASKRSRGFGFVTFSSMAEVDAAMAARPHSIDGRVVEPKRAVAREESGKPGAHVTVKKLFVGGIKEDTEEHHLRDYFEEYGKIDTIEIITDRQSGKKRGFGFVTFDDHDPVDKIVLQKYHTINGHNAEVRKALSRQEMQEVQSSRSGRGGNFGFGDSRGGGGNFGPGPGSNFRGGSDGYGSGRGFGDGYNGYGGGPGGNYGSGSYNDFGNYNQQPSNYGPMKSGNFGGSRNMGGPYGGGNYGPGGSGGSGGYGGRSRY

SEQ ID NO: 5 - DNA, 21 bp, Artifical sequence
gaggaaauuauggaaguggtt

SEQ ID NO: 6 - DNA, 21 bp, Artifical sequence
ccacuuccauaauuuccucct

SEQ ID NO: 7 - DNA, 21 bp, Artifical sequence
cuuuggugguagcaggaactt

SEQ ID NO: 8 - DNA, 21 bp, Artifical sequence
guuccugcuaccaccaaagtt

SEQ ID NO: 9 - DNA, 21 bp, Artifical sequence
uucuccgaacgugucacgutt

SEQ ID NO: 10 - DNA, 21 bp, Artifical sequence
acgugacacguucggagaatt